European Patent Specification EP 3 737 744 B1, published March 26, 2025. Title: GENETICALLY ENGINEERED HEMATOPOIETIC STEM CELL AS A PLATFORM FOR SYSTEMIC PROTEIN EXPRESSION. Applicant: GENETHON UNIVERSITE D'EVRY-VAL-D'ESSONNE Institut National de la Sante et de la Recherche Medicale (INSERM). The sequence listing filed with the application follows.

SEQUENCE LISTING (68 sequences)

SEQ ID NO: 1 - DNA, 20 bp, Artificial Sequence
  Partial nucleic acid sequence of HBA 4
  Partial nucleic acid sequence of HBA 4
ggggcgcggcctggaccgca

SEQ ID NO: 2 - DNA, 23 bp, Artificial Sequence
  Full nucleic acid sequence of HBA 4
  Full nucleic acid sequence of HBA 4
ggggcgcggcctggaccgcaggg

SEQ ID NO: 3 - DNA, 20 bp, Artificial Sequence
  Partial nucleic acid sequence of HBA 10
  Partial nucleic acid sequence of HBA 10
gggtttatgcttggggcgcg

SEQ ID NO: 4 - DNA, 23 bp, Artificial Sequence
  Full nucleic acid sequence of HBA 10
  Full nucleic acid sequence of HBA 10
gggtttatgcttggggcgcgggg

SEQ ID NO: 5 - DNA, 20 bp, Artificial Sequence
  Partial nucleic acid sequence of HBA 12
  Partial nucleic acid sequence of HBA 12
gactcagagagaacccacca

SEQ ID NO: 6 - DNA, 23 bp, Artificial Sequence
  Full nucleic acid sequence of HBA 12
  Full nucleic acid sequence of HBA 12
gactcagagagaacccaccatgg

SEQ ID NO: 7 - DNA, 20 bp, Artificial Sequence
  Partial nucleic acid sequence of HBA 14
  Partial nucleic acid sequence of HBA 14
tgggttctctctgagtctgt

SEQ ID NO: 8 - DNA, 23 bp, Artificial Sequence
  Full nucleic acid sequence of HBA 14
  Full nucleic acid sequence of HBA 14
tgggttctctctgagtctgtggg

SEQ ID NO: 9 - DNA, 20 bp, Artificial Sequence
  Partial nucleic acid sequence of HBA 19.1
  Partial nucleic acid sequence of HBA 19.1
gcgcgggggcacgcccggcc

SEQ ID NO: 10 - DNA, 23 bp, Artificial Sequence
  Full nucleic acid sequence of HBA 19.1
  Full nucleic acid sequence of HBA 19.1
gcgcgggggcacgcccggccggg

SEQ ID NO: 11 - DNA, 20 bp, Artificial Sequence
  Partial nucleic acid sequence of HBA 15.1
  Partial nucleic acid sequence of HBA 15.1
gggttctctctgagtctgtg

SEQ ID NO: 12 - DNA, 23 bp, Artificial Sequence
  Full nucleic acid sequence of HBA 15.1
  Full nucleic acid sequence of HBA 15.1
gggttctctctgagtctgtgggg

SEQ ID NO: 13 - DNA, 20 bp, Artificial Sequence
  Partial nucleic acid sequence of HBA 16.1
  Partial nucleic acid sequence of HBA 16.1
gtcggcaggagacagcacca

SEQ ID NO: 14 - DNA, 23 bp, Artificial Sequence
  Full nucleic acid sequence of HBA 16.1
  Full nucleic acid sequence of HBA 16.1
gtcggcaggagacagcaccatgg

SEQ ID NO: 15 - DNA, 20 bp, Artificial Sequence
  Partial nucleic acid sequence of HBA 17-G
  Partial nucleic acid sequence of HBA 17-G
gcaggagacagcaccatggt

SEQ ID NO: 16 - DNA, 23 bp, Artificial Sequence
  Full nucleic acid sequence of HBA 17-G
  Full nucleic acid sequence of HBA 17-G
gcaggagacagcaccatggtggg

SEQ ID NO: 17 - DNA, 20 bp, Artificial Sequence
  Partial nucleic acid sequence of HBA 20.1
  Partial nucleic acid sequence of HBA 20.1
cataaaccctggcgcgctcg

SEQ ID NO: 18 - DNA, 23 bp, Artificial Sequence
  Full nucleic acid sequence of HBA 20.1
  Full nucleic acid sequence of HBA 20.1
cataaaccctggcgcgctcgcgg

SEQ ID NO: 19 - DNA, 20 bp, Artificial Sequence
  Partial nucleic acid sequence of HBA 5.1
  Partial nucleic acid sequence of HBA 5.1
ttgaatgctccagccggttc

SEQ ID NO: 20 - DNA, 23 bp, Artificial Sequence
  Full nucleic acid sequence of HBA 5.1
  Full nucleic acid sequence of HBA 5.1
ttgaatgctccagccggttccag

SEQ ID NO: 21 - DNA, 20 bp, Artificial Sequence
  Partial nucleic acid sequence of gRNA2
  Partial nucleic acid sequence of gRNA2
cgggaggcttcgcccaatcc

SEQ ID NO: 22 - DNA, 23 bp, Artificial Sequence
  Full nucleic acid sequence of gRNA2
  Full nucleic acid sequence of gRNA2
cgggaggcttcgcccaatcctgg

SEQ ID NO: 23 - DNA, 20 bp, Artificial Sequence
  Partial nucleic acid sequence of gRNA3
  Partial nucleic acid sequence of gRNA3
cgggcgagcgagtgcgagcc

SEQ ID NO: 24 - DNA, 22 bp, Artificial Sequence
  Full nucleic acid sequence of gRNA3
  Full nucleic acid sequence of gRNA3
cgggcgagcgagtgcgagccgg

SEQ ID NO: 25 - DNA, 20 bp, Artificial Sequence
  Partial nucleic acid sequence of gRNA11
  Partial nucleic acid sequence of gRNA11
gggaggcttcgcccaatcct

SEQ ID NO: 26 - DNA, 23 bp, Artificial Sequence
  Full nucleic acid sequence of gRNA11
  Full nucleic acid sequence of gRNA11
gggaggcttcgcccaatcctggg

SEQ ID NO: 27 - DNA, 20 bp, Artificial Sequence
  Partial nucleic acid sequence of HBA INT1 72.1
  Partial nucleic acid sequence of HBA INT1 72.1
caggccaccctcaaccgtcc

SEQ ID NO: 28 - DNA, 23 bp, Artificial Sequence
  Full nucleic acid sequence of HBA INT1 72.1
  Full nucleic acid sequence of HBA INT1 72.1
caggccaccctcaaccgtcctgg

SEQ ID NO: 29 - DNA, 20 bp, Artificial Sequence
  Partial nucleic acid sequence of HBA INT1 73.2
  Partial nucleic acid sequence of HBA INT1 73.2
tccggggccaggacggttga

SEQ ID NO: 30 - DNA, 23 bp, Artificial Sequence
  Full nucleic acid sequence of HBA INT1 73.2
  Full nucleic acid sequence of HBA INT1 73.2
tccggggccaggacggttgaggg

SEQ ID NO: 31 - DNA, 20 bp, Artificial Sequence
  Partial nucleic acid sequence of HBA INT1 73b.1
  Partial nucleic acid sequence of HBA INT1 73b.1
gtccggggccaggacggttg

SEQ ID NO: 32 - DNA, 23 bp, Artificial Sequence
  Full nucleic acid sequence of HBA INT1 73b.1
  Full nucleic acid sequence of HBA INT1 73b.1
gtccggggccaggacggttgagg

SEQ ID NO: 33 - DNA, 20 bp, Artificial Sequence
  Partial nucleic acid sequence of HBA INT2 13.2
  Partial nucleic acid sequence of HBA INT2 13.2
ccctcgacccagatcgctcc

SEQ ID NO: 34 - DNA, 23 bp, Artificial Sequence
  Full nucleic acid sequence of HBA INT2 13.2
  Full nucleic acid sequence of HBA INT2 13.2
ccctcgacccagatcgctcccgg

SEQ ID NO: 35 - DNA, 20 bp, Artificial Sequence
  Partial nucleic acid sequence of HBA INT2 63.2
  Partial nucleic acid sequence of HBA INT2 63.2
gaagagggtcagtgcggccc

SEQ ID NO: 36 - DNA, 23 bp, Artificial Sequence
  Full nucleic acid sequence of HBA INT2 63.2
  Full nucleic acid sequence of HBA INT2 63.2
gaagagggtcagtgcggcccagg

SEQ ID NO: 37 - DNA, 20 bp, Artificial Sequence
  Partial nucleic acid sequence of HBA INT2 74.1
  Partial nucleic acid sequence of HBA INT2 74.1
gcgtgatcctctgccctgag

SEQ ID NO: 38 - DNA, 23 bp, Artificial Sequence
  Full nucleic acid sequence of HBA INT2 74.1
  Full nucleic acid sequence of HBA INT2 74.1
gcgtgatcctctgccctgagagg

SEQ ID NO: 39 - DNA, 20 bp, Artificial Sequence
  Partial nucleic acid sequence of HBB 37.1
  Partial nucleic acid sequence of HBB 37.1
gggttggccaatctactccc

SEQ ID NO: 40 - DNA, 22 bp, Artificial Sequence
  Full nucleic acid sequence of HBB 37.1
  Full nucleic acid sequence of HBB 37.1
ggttggccaatctactcccagg

SEQ ID NO: 41 - DNA, 20 bp, Artificial Sequence
  Partial nucleic acid sequence of HBB 49.2
  Partial nucleic acid sequence of HBB 49.2
gggttggccaatctactccc

SEQ ID NO: 42 - DNA, 23 bp, Artificial Sequence
  Full nucleic acid sequence of HBB 49.2
  Full nucleic acid sequence of HBB 49.2
gggttggccaatctactcccagg

SEQ ID NO: 43 - DNA, 20 bp, Artificial Sequence
  Partial nucleic acid sequence of HBB 53.1
  Partial nucleic acid sequence of HBB 53.1
ggagtagattggccaaccct

SEQ ID NO: 44 - DNA, 23 bp, Artificial Sequence
  Full nucleic acid sequence of HBB 53.1
  Full nucleic acid sequence of HBB 53.1
ggagtagattggccaaccctagg

SEQ ID NO: 45 - DNA, 20 bp, Artificial Sequence
  Partial nucleic acid sequence of HBB 54.1
  Partial nucleic acid sequence of HBB 54.1
gattggccaaccctagggtg

SEQ ID NO: 46 - DNA, 23 bp, Artificial Sequence
  Full nucleic acid sequence of HBB 54.1
  Full nucleic acid sequence of HBB 54.1
gattggccaaccctagggtgtgg

SEQ ID NO: 47 - DNA, 20 bp, Artificial Sequence
  Partial nucleic acid sequence of HBB 77.1
  Partial nucleic acid sequence of HBB 77.1
gagtagattggccaacccta

SEQ ID NO: 48 - DNA, 23 bp, Artificial Sequence
  Full nucleic acid sequence of HBB 77.1
  Full nucleic acid sequence of HBB 77.1
gagtagattggccaaccctaggg

SEQ ID NO: 49 - DNA, 20 bp, Artificial Sequence
  Partial nucleic acid sequence of HBB INT 1 36.2
  Partial nucleic acid sequence of HBB INT 1 36.2
tggtatcaaggttacaagac

SEQ ID NO: 50 - DNA, 23 bp, Artificial Sequence
  Full nucleic acid sequence of HBB INT 1 36.2
  Full nucleic acid sequence of HBB INT 1 36.2
tggtatcaaggttacaagacagg

SEQ ID NO: 51 - DNA, 20 bp, Artificial Sequence
  Partial nucleic acid sequence of HBB INT1 36.2 REV
  Partial nucleic acid sequence of HBB INT1 36.2 REV
tccacatgcccagtttctat

SEQ ID NO: 52 - DNA, 23 bp, Artificial Sequence
  Full nucleic acid sequence of HBB INT1 36.2 REV
  Full nucleic acid sequence of HBB INT1 36.2 REV
tccacatgcccagtttctattgg

SEQ ID NO: 53 - DNA, 20 bp, Artificial Sequence
  Partial nucleic acid sequence of HBB INT1 47.1
  Partial nucleic acid sequence of HBB INT1 47.1
ttaaggagaccaatagaaac

SEQ ID NO: 54 - DNA, 23 bp, Artificial Sequence
  Full nucleic acid sequence of HBB INT1 47.1
  Full nucleic acid sequence of HBB INT1 47.1
ttaaggagaccaatagaaactgg

SEQ ID NO: 55 - DNA, 20 bp, Artificial Sequence
  Partial nucleic acid sequence of HBB INT1 48.1
  Partial nucleic acid sequence of HBB INT1 48.1
taaggagaccaatagaaact

SEQ ID NO: 56 - DNA, 23 bp, Artificial Sequence
  Full nucleic acid sequence of HBB INT1 48.1
  Full nucleic acid sequence of HBB INT1 48.1
taaggagaccaatagaaactggg

SEQ ID NO: 57 - DNA, 20 bp, Artificial Sequence
  Partial nucleic acid sequence of HBB INT2 340.1
  Partial nucleic acid sequence of HBB INT2 340.1
ctgcctagtacattactatt

SEQ ID NO: 58 - DNA, 23 bp, Artificial Sequence
  Full nucleic acid sequence of HBB INT2 340.1
  Full nucleic acid sequence of HBB INT2 340.1
ctgcctagtacattactatttgg

SEQ ID NO: 59 - DNA, 20 bp, Artificial Sequence
  Partial nucleic acid sequence of HBB INT2 797.1
  Partial nucleic acid sequence of HBB INT2 797.1
attagcaaaagggcctagct

SEQ ID NO: 60 - DNA, 23 bp, Artificial Sequence
  Full nucleic acid sequence of HBB INT2 797.1
  Full nucleic acid sequence of HBB INT2 797.1
attagcaaaagggcctagcttgg

SEQ ID NO: 61 - DNA, 20 bp, Artificial Sequence
  Partial nucleic acid sequence of HBB INT2 20.1
  Partial nucleic acid sequence of HBB INT2 20.1
gttaagttcatgtcatagga

SEQ ID NO: 62 - DNA, 23 bp, Artificial Sequence
  Full nucleic acid sequence of HBB INT2 20.1
  Full nucleic acid sequence of HBB INT2 20.1
gttaagttcatgtcataggaagg

SEQ ID NO: 63 - DNA, 20 bp, Artificial Sequence
  Partial nucleic acid sequence of HBB INT2 39.2
  Partial nucleic acid sequence of HBB INT2 39.2
gacgaatgattgcatcagtg

SEQ ID NO: 64 - DNA, 23 bp, Artificial Sequence
  Full nucleic acid sequence of HBB INT2 39.2
  Full nucleic acid sequence of HBB INT2 39.2
gacgaatgattgcatcagtgtgg

SEQ ID NO: 65 - DNA, 20 bp, Artificial Sequence
  Partial nucleic acid sequence of an HBB gRNA
cttgccccacagggcagtaa

SEQ ID NO: 66 - DNA, 23 bp, Artificial Sequence
  Full nucleic acid sequence of a HBB gRNA
cttgccccacagggcagtaacgg

SEQ ID NO: 67 - DNA, 20 bp, Artificial Sequence
  partial nucleic acid sequence of an AAVS1 gRNA
gtcccctccaccccacagtg

SEQ ID NO: 68 - DNA, 23 bp, Artificial Sequence
  Full nucleic acid sequence of a AAVS1 gRNA
gtcccctccaccccacagtgggg